European Patent Application EP 4 610 659 A2, published September 3, 2025. Title: MAMMALIAN MHC PEPTIDE DISPLAY AS AN EPITOPE SELECTION TOOL FOR VACCINE DESIGN. Applicant: ETH Zurich. Application EP. The sequence listing filed with the application follows.

SEQUENCE LISTING (26 sequences)

SEQ ID NO: 1 - protein, 18 aa, Mammalia
  REGION 1..18: note = Human MHC molecule
LKREITFHGAKEISLSYS

SEQ ID NO: 2 - protein, 15 aa, Mammalia
  REGION 1..15: note = Human MHC molecule
LKREITFHGAKEISL

SEQ ID NO: 3 - protein, 15 aa, Mammalia
  REGION 1..15: note = Human MHC molecule
KREITFHGAKEISLS

SEQ ID NO: 4 - protein, 15 aa, Mammalia
  REGION 1..15: note = Human MHC molecule
REITFHGAKEISLSY

SEQ ID NO: 5 - protein, 15 aa, Mammalia
  REGION 1..15: note = Human MHC molecule
EITFHGAKEISLSYS

SEQ ID NO: 6 - protein, 15 aa, Mammalia
  REGION 1..15: note = Human MHC molecule
LKREITFHGAKEISL

SEQ ID NO: 7 - protein, 15 aa, Mammalia
  REGION 1..15: note = Human MHC molecule
EITFHGAKEISLSYS

SEQ ID NO: 8 - protein, 15 aa, Mammalia
  REGION 1..15: note = Human MHC molecule
REITFHGAKEISLSY

SEQ ID NO: 9 - protein, 15 aa, Mammalia
  REGION 1..15: note = Human MHC molecule
KREITFHGAKEISLS

SEQ ID NO: 10 - protein, 15 aa, Mammalia
  REGION 1..15: note = Human MHC molecule
LKREITFHGAKEISL

SEQ ID NO: 11 - protein, 15 aa, Mammalia
  REGION 1..15: note = Human MHC molecule
KREITFHGAKEISLS

SEQ ID NO: 12 - protein, 15 aa, Mammalia
  REGION 1..15: note = Human MHC molecule
REITFHGAKEISLSY

SEQ ID NO: 13 - protein, 15 aa, Mammalia
  REGION 1..15: note = Human MHC molecule
EITFHGAKEISLSYS

SEQ ID NO: 14 - protein, 18 aa, Mammalia
  REGION 1..18: note = Human MHC molecule
YRKLKREITFHGAKEISL

SEQ ID NO: 15 - protein, 18 aa, Mammalia
  REGION 1..18: note = Human MHC molecule
RKLKREITFHGAKEISLS

SEQ ID NO: 16 - protein, 18 aa, Mammalia
  REGION 1..18: note = Human MHC molecule
KLKREITFHGAKEISLSY

SEQ ID NO: 17 - protein, 18 aa, Mammalia
  REGION 1..18: note = Human MHC molecule
LKREITFHGAKEISLSYS

SEQ ID NO: 18 - protein, 12 aa, Mammalia
  REGION 1..12: note = Human MHC molecule
SVLSKFHGLFGI

SEQ ID NO: 19 - protein, 12 aa, Mammalia
  REGION 1..12: note = Human MHC molecule
GSSRRSISVFFV

SEQ ID NO: 20 - protein, 12 aa, Mammalia
  REGION 1..12: note = Human MHC molecule
LIRTTLFYVQVF

SEQ ID NO: 21 - protein, 12 aa, Mammalia
  REGION 1..12: note = Human MHC molecule
YYYFRETLMCNW

SEQ ID NO: 22 - protein, 12 aa, Mammalia
  REGION 1..12: note = Human MHC molecule
RSLKFTVVCLGA

SEQ ID NO: 23 - protein, 12 aa, Mammalia
  REGION 1..12: note = Human MHC molecule
YSWTWVFFACGG

SEQ ID NO: 24 - protein, 12 aa, Mammalia
  REGION 1..12: note = Human MHC molecule
VTLINRRVEWRL

SEQ ID NO: 25 - protein, 12 aa, Mammalia
  REGION 1..12: note = Human MHC molecule
ASWTWVFFACGG

SEQ ID NO: 26 - protein, 12 aa, Mammalia
  REGION 1..12: note = Human MHC molecule
YHYRALSYIVTY